European Patent Specification EP 3 565 592 B1, published March 1, 2023. Title: METHODS FOR TREATING METABOLIC DISEASES BY INHIBITING MYOSTATIN ACTIVATION. Applicant: Scholar Rock, Inc. Application Not Yet Assigned. The sequence listing filed with the application follows.

SEQUENCE LISTING (118 sequences)

SEQ ID NO: 1 - protein, 6 aa, Artificial Sequence
  Synthetic Polypeptide
SSYGMH

SEQ ID NO: 2 - protein, 10 aa, Artificial Sequence
  Synthetic Polypeptide
GFTFSSYGMH

SEQ ID NO: 3 - protein, 10 aa, Artificial Sequence
  Synthetic Polypeptide
GFAFSSYGMH

SEQ ID NO: 4 - protein, 17 aa, Artificial Sequence
  Synthetic Polypeptide
VISYDGSNKYYADSVKG

SEQ ID NO: 5 - protein, 7 aa, Artificial Sequence
  Synthetic Polypeptide
ISYDGSN

SEQ ID NO: 6 - protein, 17 aa, Artificial Sequence
  Synthetic Polypeptide
VISYDGSIKYYADSVKG

SEQ ID NO: 7 - protein, 7 aa, Artificial Sequence
  Synthetic Polypeptide
ISYDGSI

SEQ ID NO: 8 - protein, 17 aa, Artificial Sequence
  Synthetic Polypeptide
VISYDGNNKYYADSVKG

SEQ ID NO: 9 - protein, 7 aa, Artificial Sequence
  Synthetic Polypeptide
ISYDGNN

SEQ ID NO: 10 - protein, 17 aa, Artificial Sequence
  Synthetic Polypeptide
DLLVRFLEWSHYYGMDV

SEQ ID NO: 11 - protein, 17 aa, Artificial Sequence
  Synthetic Polypeptide
DLLVRFLEWSHKYGMDV

SEQ ID NO: 12 - protein, 13 aa, Artificial Sequence
  Synthetic Polypeptide
SGSSSNIGSNTVH

SEQ ID NO: 13 - protein, 8 aa, Artificial Sequence
  Synthetic Polypeptide
SSNIGSNT

SEQ ID NO: 14 - protein, 13 aa, Artificial Sequence
  Synthetic Polypeptide
SGSTSNIGSNTVH

SEQ ID NO: 15 - protein, 8 aa, Artificial Sequence
  Synthetic Polypeptide
TSNIGSNT

SEQ ID NO: 16 - protein, 13 aa, Artificial Sequence
  Synthetic Polypeptide
SGSSSNIGGNTVH

SEQ ID NO: 17 - protein, 8 aa, Artificial Sequence
  Synthetic Polypeptide
SSNIGGNT

SEQ ID NO: 18 - protein, 7 aa, Artificial Sequence
  Synthetic Polypeptide
SDNQRPS

SEQ ID NO: 19 - protein, 3 aa, Artificial Sequence
  Synthetic Polypeptide
SDN

SEQ ID NO: 20 - protein, 7 aa, Artificial Sequence
  Synthetic Polypeptide
SDDQRPS

SEQ ID NO: 21 - protein, 3 aa, Artificial Sequence
  Synthetic Polypeptide
SDD

SEQ ID NO: 22 - protein, 10 aa, Artificial Sequence
  Synthetic Polypeptide
AAWDDSLNGV

SEQ ID NO: 23 - protein, 10 aa, Artificial Sequence
  Synthetic Polypeptide
AAWDESLNGV

SEQ ID NO: 24 - protein, 126 aa, Artificial Sequence
  Synthetic Polypeptide
QIQLVQSGGGVVQPGRSLRLSCAASGFTFSSYGMHWVRQAPGKGLEWVAVISYDGSNKYYADSVKGRFTISRDNSKNTLYLQMNSLRAEDTAVYYCARDLLVRFLEWSHYYGMDVWGQGTTVTVSS

SEQ ID NO: 25 - protein, 126 aa, Artificial Sequence
  Synthetic Polypeptide
QVQLVESGGGVVQPGRSLRLSCAASGFTFSSYGMHWVRQAPGKGLEWVAVISYDGSNKYYADSVKGRFTISRDNSKNTLYLQMNSLRAEDTAVYYCARDLLVRFLEWSHYYGMDVWGQGTTVTVSS

SEQ ID NO: 26 - protein, 126 aa, Artificial Sequence
  Synthetic Polypeptide
QIQLVQSGGGVVQPGRSLRLSCAASGFAFSSYGMHWVRQAPGKGLEWVAVISYDGSIKYYADSVKGRFTISRDNSKNTLYLQMNSLRAEDTAVYYCARDLLVRFLEWSHKYGMDVWGQGTTVTVSS

SEQ ID NO: 27 - protein, 126 aa, Artificial Sequence
  Synthetic Polypeptide
QVQLVESGGGVVQPGRSLRLSCAASGFAFSSYGMHWVRQAPGKGLEWVAVISYDGSIKYYADSVKGRFTISRDNSKNTLYLQMNSLRAEDTAVYYCARDLLVRFLEWSHKYGMDVWGQGTTVTVSS

SEQ ID NO: 28 - protein, 126 aa, Artificial Sequence
  Synthetic Polypeptide
QIQLVQSGGGVVQPGRSLRLSCAASGFAFSSYGMHWVRQAPGKGLEWVAVISYDGNNKYYADSVKGRFTISRDNSKNTLYLQMNSLRAEDTAVYYCARDLLVRFLEWSHKYGMDVWGQGTTVTVSS

SEQ ID NO: 29 - protein, 126 aa, Artificial Sequence
  Synthetic Polypeptide
QVQLVESGGGVVQPGRSLRLSCAASGFAFSSYGMHWVRQAPGKGLEWVAVISYDGNNKYYADSVKGRFTISRDNSKNTLYLQMNSLRAEDTAVYYCARDLLVRFLEWSHKYGMDVWGQGTTVTVSS

SEQ ID NO: 30 - protein, 109 aa, Artificial Sequence
  Synthetic Polypeptide
QPVLTQPPSASGTPGQRVTISCSGSSSNIGSNTVHWYQQLPGTAPKLLIYSDNQRPSGVPDRFSGSKSGTSASLVISGLQSDDEADYYCAAWDDSLNGVFGGGTKLTVL

SEQ ID NO: 31 - protein, 109 aa, Artificial Sequence
  Synthetic Polypeptide
QSVLTQPPSASGTPGQRVTISCSGSSSNIGSNTVHWYQQLPGTAPKLLIYSDNQRPSGVPDRFSGSKSGTSASLAISGLQSEDEADYYCAAWDDSLNGVFGGGTKLTVL

SEQ ID NO: 32 - protein, 109 aa, Artificial Sequence
  Synthetic Polypeptide
QPVLTQPPSASGTPGQRVTISCSGSTSNIGSNTVHWYQQLPGTAPKLLIYSDDQRPSGVPDRFSGSKSGTSASLVISGLQSDDEADYYCAAWDESLNGVFGGGTKLTVL

SEQ ID NO: 33 - protein, 109 aa, Artificial Sequence
  Synthetic Polypeptide
QSVLTQPPSASGTPGQRVTISCSGSTSNIGSNTVHWYQQLPGTAPKLLIYSDDQRPSGVPDRFSGSKSGTSASLAISGLQSEDEADYYCAAWDESLNGVFGGGTKLTVL

SEQ ID NO: 34 - protein, 109 aa, Artificial Sequence
  Synthetic Polypeptide
QPVLTQPPSASGTPGQRVTISCSGSSSNIGGNTVHWYQQLPGTAPKLLIYSDDQRPSGVPDRFSGSKSGTSASLVISGLQSDDEADYYCAAWDESLNGVFGGGTKLTVL

SEQ ID NO: 35 - protein, 109 aa, Artificial Sequence
  Synthetic Polypeptide
QSVLTQPPSASGTPGQRVTISCSGSSSNIGGNTVHWYQQLPGTAPKLLIYSDDQRPSGVPDRFSGSKSGTSASLAISGLQSEDEADYYCAAWDESLNGVFGGGTKLTVL

SEQ ID NO: 36 - protein, 98 aa, Artificial Sequence
  Synthetic Polypeptide
QVQLVESGGGVVQPGRSLRLSCAASGFTFSSYGMHWVRQAPGKGLEWVAVISYDGSNKYYADSVKGRFTISRDNSKNTLYLQMNSLRAEDTAVYYCAR

SEQ ID NO: 37 - protein, 98 aa, Artificial Sequence
  Synthetic Polypeptide
QSVLTQPPSASGTPGQRVTISCSGSSSNIGSNTVNWYQQLPGTAPKLLIYSNNQRPSGVPDRFSGSKSGTSASLAISGLQSEDEADYYCAAWDDSLNG

SEQ ID NO: 38 - DNA, 378 bp, Artificial Sequence
  Synthetic Polynucleotide
cagatccagctggtgcagtctgggggaggcgtggtccagcctgggaggtccctgagactctcctgtgcagcgtctggattcaccttcagtagctatggcatgcactgggtccgccaggctccaggcaaggggctggagtgggtggcagttatatcatatgatggaagtaataaatactatgcagactccgtgaagggccgattcaccatctccagagacaattccaagaacacgctgtatctgcaaatgaacagcctgagagccgaggacacggctgtgtattactgtgcgagagatctcctggtgcgatttttggagtggtcgcactactacggtatggacgtctggggccaagggaccacggtcaccgtctcctca

SEQ ID NO: 39 - DNA, 378 bp, Artificial Sequence
  Synthetic Polynucleotide
caggtgcagctggtggagtctgggggaggcgtggtccagcctgggaggtccctgagactctcctgtgcagcgtctggattcaccttcagtagctatggcatgcactgggtccgccaggctccaggcaaggggctggagtgggtggcagttatatcatatgatggaagtaataaatactatgcagactccgtgaagggccgattcaccatctccagagacaattccaagaacacgctgtatctgcaaatgaacagcctgagagccgaggacacggctgtgtattactgtgcgagagatctcctggtgcgatttttggagtggtcgcactactacggtatggacgtctggggccaagggaccacggtcaccgtctcctca

SEQ ID NO: 40 - DNA, 378 bp, Artificial Sequence
  Synthetic Polynucleotide
cagatccagctggtgcagtctgggggaggcgtggtccagcctgggaggtccctgagactctcctgtgcagcgtctggattcgccttcagtagctatggcatgcactgggtccgccaggctccaggcaaggggctggagtgggtggcagttatatcatatgatggaagtatcaaatactatgcagactccgtgaagggccgattcaccatctccagagacaattccaagaacacgctgtatctgcaaatgaacagcctgagagccgaggacacggctgtgtattactgtgcgagagatctcctggtgcgatttttggagtggtcgcacaagtacggtatggacgtctggggccaagggaccacggtcaccgtctcctca

SEQ ID NO: 41 - DNA, 378 bp, Artificial Sequence
  Synthetic Polynucleotide
caggtgcagctggtggagtctgggggaggcgtggtccagcctgggaggtccctgagactctcctgtgcagcgtctggattcgccttcagtagctatggcatgcactgggtccgccaggctccaggcaaggggctggagtgggtggcagttatatcatatgatggaagtatcaaatactatgcagactccgtgaagggccgattcaccatctccagagacaattccaagaacacgctgtatctgcaaatgaacagcctgagagccgaggacacggctgtgtattactgtgcgagagatctcctggtgcgatttttggagtggtcgcacaagtacggtatggacgtctggggccaagggaccacggtcaccgtctcctca

SEQ ID NO: 42 - DNA, 378 bp, Artificial Sequence
  Synthetic Polynucleotide
cagatccagctggtgcagtctgggggaggcgtggtccagcctgggaggtccctgagactctcctgtgcagcgtctggattcgccttcagtagctatggcatgcactgggtccgccaggctccaggcaaggggctggagtgggtggcagttatatcatatgatggaaataataaatactatgcagactccgtgaagggccgattcaccatctccagagacaattccaagaacacgctgtatctgcaaatgaacagcctgagagccgaggacacggctgtgtattactgtgcgagagatctcctggtgcgatttttggagtggtcgcacaagtacggtatggacgtctggggccaagggaccacggtcaccgtctcctca

SEQ ID NO: 43 - DNA, 378 bp, Artificial Sequence
  Synthetic Polynucleotide
caggtgcagctggtggagtctgggggaggcgtggtccagcctgggaggtccctgagactctcctgtgcagcgtctggattcgccttcagtagctatggcatgcactgggtccgccaggctccaggcaaggggctggagtgggtggcagttatatcatatgatggaaataataaatactatgcagactccgtgaagggccgattcaccatctccagagacaattccaagaacacgctgtatctgcaaatgaacagcctgagagccgaggacacggctgtgtattactgtgcgagagatctcctggtgcgatttttggagtggtcgcacaagtacggtatggacgtctggggccaagggaccacggtcaccgtctcctca

SEQ ID NO: 44 - DNA, 327 bp, Artificial Sequence
  Synthetic Polynucleotide
cagcctgtgctgactcagccaccctcagcgtctgggacccccgggcagagggtcaccatctcttgttctggaagcagctccaacatcggaagtaatactgtccactggtaccagcaactcccaggaacggcccccaaactcctcatctatagtgataatcagcgcccctcaggggtccctgaccgattctctggctccaagtctggcacctcagcctccctggtcatcagtgggctccagtctgacgatgaggctgattattactgtgcagcatgggatgacagcctgaatggggtgttcggcggagggaccaagctgaccgtccta

SEQ ID NO: 45 - DNA, 327 bp, Artificial Sequence
  Synthetic Polynucleotide
cagtctgtgctgactcagccaccctcagcgtctgggacccccgggcagagggtcaccatctcttgttctggaagcagctccaacatcggaagtaatactgtccactggtaccagcaactcccaggaacggcccccaaactcctcatctatagtgataatcagcgcccctcaggggtccctgaccgattctctggctccaagtctggcacctcagcctccctggccatcagtgggctccagtctgaggatgaggctgattattactgtgcagcatgggatgacagcctgaatggggtgttcggcggagggaccaagctgaccgtccta

SEQ ID NO: 46 - DNA, 327 bp, Artificial Sequence
  Synthetic Polynucleotide
cagcctgtgctgactcagccaccctcagcgtctgggacccccgggcagagggtcaccatctcttgttctggaagcacctccaacatcggaagtaatactgtccactggtaccagcaactcccaggaacggcccccaaactcctcatctatagtgatgatcagcgcccctcaggggtccctgaccgattctctggctccaagtctggcacctcagcctccctggtcatcagtgggctccagtctgacgatgaggctgattattactgtgcagcatgggatgagagcctgaatggggtgttcggcggagggaccaagctgaccgtccta

SEQ ID NO: 47 - DNA, 327 bp, Artificial Sequence
  Synthetic Polynucleotide
cagtctgtgctgactcagccaccctcagcgtctgggacccccgggcagagggtcaccatctcttgttctggaagcacctccaacatcggaagtaatactgtccactggtaccagcaactcccaggaacggcccccaaactcctcatctatagtgatgatcagcgcccctcaggggtccctgaccgattctctggctccaagtctggcacctcagcctccctggccatcagtgggctccagtctgaggatgaggctgattattactgtgcagcatgggatgagagcctgaatggggtgttcggcggagggaccaagctgaccgtccta

SEQ ID NO: 48 - DNA, 327 bp, Artificial Sequence
  Synthetic Polynucleotide
cagcctgtgctgactcagccaccctcagcgtctgggacccccgggcagagggtcaccatctcttgttctggaagcagctccaacatcggaggaaatactgtccactggtaccagcaactcccaggaacggcccccaaactcctcatctatagtgatgatcagcgcccctcaggggtccctgaccgattctctggctccaagtctggcacctcagcctccctggtcatcagtgggctccagtctgacgatgaggctgattattactgtgcagcatgggatgagagcctgaatggggtgttcggcggagggaccaagctgaccgtccta

SEQ ID NO: 49 - DNA, 327 bp, Artificial Sequence
  Synthetic Polynucleotide
cagtctgtgctgactcagccaccctcagcgtctgggacccccgggcagagggtcaccatctcttgttctggaagcagctccaacatcggaggaaatactgtccactggtaccagcaactcccaggaacggcccccaaactcctcatctatagtgatgatcagcgcccctcaggggtccctgaccgattctctggctccaagtctggcacctcagcctccctggccatcagtgggctccagtctgaggatgaggctgattattactgtgcagcatgggatgagagcctgaatggggtgttcggcggagggaccaagctgaccgtccta

SEQ ID NO: 50 - protein, 452 aa, Artificial Sequence
  Synthetic Polypeptide
QVQLVESGGGVVQPGRSLRLSCAASGFTFSSYGMHWVRQAPGKGLEWVAVISYDGSNKYYADSVKGRFTISRDNSKNTLYLQMNSLRAEDTAVYYCARDLLVRFLEWSHYYGMDVWGQGTTVTVSSASTKGPSVFPLAPCSRSTSESTAALGCLVKDYFPEPVTVSWNSGALTSGVHTFPAVLQSSGLYSLSSVVTVPSSSLGTKTYTCNVDHKPSNTKVDKRVESKYGPPCPPCPAPEFLGGPSVFLFPPKPKDTLMISRTPEVTCVVVDVSQEDPEVQFNWYVDGVEVHNAKTKPREEQFNSTYRVVSVLTVLHQDWLNGKEYKCKVSNKGLPSSIEKTISKAKGQPREPQVYTLPPSQEEMTKNQVSLTCLVKGFYPSDIAVEWESNGQPENNYKTTPPVLDSDGSFFLYSRLTVDKSRWQEGNVFSCSVMHEALHNHYTQKSLSLSLG

SEQ ID NO: 51 - protein, 215 aa, Artificial Sequence
  Synthetic Polypeptide
QSVLTQPPSASGTPGQRVTISCSGSSSNIGSNTVHWYQQLPGTAPKLLIYSDNQRPSGVPDRFSGSKSGTSASLAISGLQSEDEADYYCAAWDDSLNGVFGGGTKLTVLGQPKAAPSVTLFPPSSEELQANKATLVCLISDFYPGAVTVAWKADSSPVKAGVETTTPSKQSNNKYAASSYLSLTPEQWKSHRSYSCQVTHEGSTVEKTVAPTECS

SEQ ID NO: 52 - protein, 352 aa, Homo sapiens [sequence omitted]

SEQ ID NO: 53 - protein, 352 aa, Rattus rattus
NEDSEREANVEKEGLCNACAWRQNTRYSRIEAIKIQILSKLRLETAPNISKDAIRQLLPRAPPLRELIDQYDVQRDDSSDGSLEDDDYHATTETIITMPTESDFLMQADGKPKCCFFKFSSKIQYNKVVKAQLWIYLRAVKTPTTVFVQILRLIKPMKDGTRYTGIRSLKLDMSPGTGIWQSIDVKTVLQNWLKQPESNLGIEIKALDENGHDLAVTFPGPGEDGLNPFLEVKVTDTPKRSRRDFGLDCDEHSTESRCCRYPLTVDFEAFGWDWIIAPKRYKANYCSGECEFVFLQKYPHTHLVHQANPRGSAGPCCTPTKMSPINMLYFNGKEQIIYGKIPAMVVDRCGCS

SEQ ID NO: 54 - protein, 352 aa, Mus musculus
NEGSEREENVEKEGLCNACAWRQNTRYSRIEAIKIQILSKLRLETAPNISKDAIRQLLPRAPPLRELIDQYDVQRDDSSDGSLEDDDYHATTETIITMPTESDFLMQADGKPKCCFFKFSSKIQYNKVVKAQLWIYLRPVKTPTTVFVQILRLIKPMKDGTRYTGIRSLKLDMSPGTGIWQSIDVKTVLQNWLKQPESNLGIEIKALDENGHDLAVTFPGPGEDGLNPFLEVKVTDTPKRSRRDFGLDCDEHSTESRCCRYPLTVDFEAFGWDWIIAPKRYKANYCSGECEFVFLQKYPHTHLVHQANPRGSAGPCCTPTKMSPINMLYFNGKEQIIYGKIPAMVVDRCGCS

SEQ ID NO: 55 - protein, 277 aa, Macaca fascicularis
NENSEQKENVEKEGLCNACTWRQNTKSSRIEAIKIQILSKLRLETAPNISKDAIRQLLPKAPPLRELIDQYDVQRDDSSDGSLEDDDYHATTETIITMPTESDFLMQVDGKPKCCFFKFSSKIQYNKVVKAQLWIYLRPVETPTTVFVQILRLIKPMKDGTRYTGIRSLKLDMNPGTGIWQSIDVKTVLQNWLKQPESNLGIEIKALDENGHDLAVTFPGPGEDGLNPFLEVKVTDTPKRSRRDFGLDCDEHSTESRCCRYPLTVDFEAFGWDWIIA

SEQ ID NO: 56 - protein, 4 aa, Artificial Sequence
  Synthetic Polypeptide
RSRR

SEQ ID NO: 57 - protein, 4 aa, Artificial Sequence
  Synthetic Polypeptide
RVRR

SEQ ID NO: 58 - protein, 5 aa, Artificial Sequence
  Synthetic Polypeptide
CPPCP

SEQ ID NO: 59 - protein, 17 aa, Artificial Sequence
  Synthetic Polypeptide
HYYGMDVWGQGTTVTVS

SEQ ID NO: 60 - protein, 89 aa, Artificial Sequence
  Synthetic Polypeptide
QSVLTQPPSASGTPGQRVTISCSGSSSNIGSNTVNWYQQLPGTAPKLLIYSNNQRPSGVPDRFSGSKSGTSASLAISGLQSEDEADYYC

SEQ ID NO: 61 - protein, 11 aa, Artificial Sequence
  Synthetic Polypeptide
VFGGGTKLTVL

SEQ ID NO: 62 - protein, 33 aa, Artificial Sequence
  Synthetic Polypeptide
PKAPPLRELIDQYDVQRDDSSDGSLEDDDYHAT

SEQ ID NO: 63 - protein, 34 aa, Artificial Sequence
  Synthetic Polypeptide
GLNPFLEVKVTDTPKRSRRDFGLDCDEHSTESRC

SEQ ID NO: 64 - protein, 80 aa, Artificial Sequence
  Synthetic Polypeptide
VDLNENSEQKENVEKEGLCNACTWRQNTKSSRIEAIKIQILSKLRLETAPNISKDVIRQLLPKAPPLRELIDQYDVQRDD

SEQ ID NO: 65 - protein, 418 aa, Artificial Sequence
  Synthetic Polypeptide
MDMRVPAQLLGLLLLWFSGVLGDYKDDDDKHHHHHHLEVLFQGPAEGPAAAAAAAAAAAAAGVGGERSSRPAPSVAPEPDGCPVCVWRQHSRELRLESIKSQILSKLRLKEAPNISREVVKQLLPKAPPLRELIDQYDVQRDDSSDGSLEDDDYHATTETIITMPTESDFLMQVDGKPKCCFFKFSSKIQYNKVVKAQLWIYLRPVETPTTVFVQILRLIKPMKDGTRYTGIRSLKLDMNPGTGIWQSIDVKTVLQNWLKQPESNLGIEIKALDENGHDLAVTFPGPGEDGLNPFLEVKVTDTPKRSRRNLGLDCDEHSSESRCCRYPLTVDFEAFGWDWIIAPKRYKANYCSGQCEYMFMQKYPHTHLVQQANPRGSAGPCCTPTKMSPINMLYFNDKQQIIYGKIPGMVVDRCGCS

SEQ ID NO: 66 - protein, 19 aa, Artificial Sequence
  Synthetic Polypeptide
ARDLLVRFLEWSHYYGMDV

SEQ ID NO: 67 - protein, 10 aa, Artificial Sequence
  Synthetic Polypeptide
AAWDDSLNGV

SEQ ID NO: 68 - protein, 128 aa, Artificial Sequence
  Synthetic Polypeptide
QIQLVQSGGGVVQPGRSLRLSCAASGFTFSSYGMHWVRQAPGKGLEWVAVISYDGSNKYYADSVKGRFTISRDNSKNTLYLQMNSLRAEDTAVYYCARDLLVRFLEWSHYYGMDVWGQGTTVTVSSGS

SEQ ID NO: 69 - protein, 125 aa, Artificial Sequence
  Synthetic Polypeptide
QPVLTQPPSASGTPGQRVTISCSGSSSNIGSNTVHWYQQLPGTAPKLLIYSDNQRPSGVPDRFSGSKSGTSASLVISGLQSDDEADYYCAAWDDSLNGVFGGGTKLTVLGQPKAAPSVTLFSPSS

SEQ ID NO: 70 - protein, 272 aa, Artificial Sequence
  Synthetic Polypeptide
QIQLVQSGGGVVQPGRSLRLSCAASGFTFSSYGMHWVRQAPGKGLEWVAVISYDGSNKYYADSVKGRFTISRDNSKNTLYLQMNSLRAEDTAVYYCARDLLVRFLEWSHYYGMDVWGQGTTVTVSSGSASAPTLGGGGSGGGGSAAAQPVLTQPPSASGTPGQRVTISCSGSSSNIGSNTVHWYQQLPGTAPKLLIYSDNQRPSGVPDRFSGSKSGTSASLVISGLQSDDEADYYCAAWDDSLNGVFGGGTKLTVLGQPKAAPSVTLFSPSS

SEQ ID NO: 71 - protein, 19 aa, Artificial Sequence
  Synthetic Polypeptide
ARESLIRFLEDPQQGGMDV

SEQ ID NO: 72 - protein, 10 aa, Artificial Sequence
  Synthetic Polypeptide
NSWTRSNNYI

SEQ ID NO: 73 - protein, 128 aa, Artificial Sequence
  Synthetic Polypeptide
QVQLQQSGAEVKKPGASVKVSCKASGYTFTSYYMHWVRQAPGQGLEWMGIINPSGGSTSYAQKFQGRVTMTRDTSTSTVYMELSSLRSEDTAVYYCARESLIRFLEDPQQGGMDVWGQGTTVTVSSGS

SEQ ID NO: 74 - protein, 126 aa, Artificial Sequence
  Synthetic Polypeptide
QSALTQPASVSGSPGQSLTISCTGTSSDIGGYNYVSWYQQHPGKAPKLIIYDVTDRPSGVSGRFSGSKSGNTASLTISGLQTEDEAEYFCNSWTRSNNYIFGGGTKLTVLGQPKAAPSVTLFPPSS

SEQ ID NO: 75 - protein, 273 aa, Artificial Sequence
  Synthetic Polypeptide
QVQLQQSGAEVKKPGASVKVSCKASGYTFTSYYMHWVRQAPGQGLEWMGIINPSGGSTSYAQKFQGRVTMTRDTSTSTVYMELSSLRSEDTAVYYCARESLIRFLEDPQQGGMDVWGQGTTVTVSSGSASAPTLGGGGSGGGGSAAAQSALTQPASVSGSPGQSLTISCTGTSSDIGGYNYVSWYQQHPGKAPKLIIYDVTDRPSGVSGRFSGSKSGNTASLTISGLQTEDEAEYFCNSWTRSNNYIFGGGTKLTVLGQPKAAPSVTLFPPSS

SEQ ID NO: 76 - protein, 15 aa, Artificial Sequence
  Synthetic Polypeptide
ARDRYSSSWGGGFDY

SEQ ID NO: 77 - protein, 10 aa, Artificial Sequence
  Synthetic Polypeptide
QSYDASSLWV

SEQ ID NO: 78 - protein, 124 aa, Artificial Sequence
  Synthetic Polypeptide
EVQLVQSGGGVVQSGRSLRLSCVASGFSFSNYGMHWVRQAPGKGLEWLAFIWYDGSNKWYADSVKGRFTISRDNSKNALYLQMNSLRAEDTAVYYCARDRYSSSWGGGFDYWGQGTVLTVSSGS

SEQ ID NO: 79 - protein, 132 aa, Artificial Sequence
  Synthetic Polypeptide
NFMLTQPHSVSESPGRTVTIPCSGRGGSIASDSVQWYQQRPGSAPTTIIYEDNQRPSGVPDRFSGSVDSSSNSASLTISGLRTEDEADYYCQSYDASSLWVFGGKTKLTVLGQPKAAPSVTLFPPSSKASGA

SEQ ID NO: 80 - protein, 275 aa, Artificial Sequence
  Synthetic Polypeptide
EVQLVQSGGGVVQSGRSLRLSCVASGFSFSNYGMHWVRQAPGKGLEWLAFIWYDGSNKWYADSVKGRFTISRDNSKNALYLQMNSLRAEDTAVYYCARDRYSSSWGGGFDYWGQGTVLTVSSGSASAPTLGGGGSGGGGSAAANFMLTQPHSVSESPGRTVTIPCSGRGGSIASDSVQWYQQRPGSAPTTIIYEDNQRPSGVPDRFSGSVDSSSNSASLTISGLRTEDEADYYCQSYDASSLWVFGGKTKLTVLGQPKAAPSVTLFPPSSKASGA

SEQ ID NO: 81 - protein, 12 aa, Artificial Sequence
  Synthetic Polypeptide
VRDRHSLGDFDY

SEQ ID NO: 82 - protein, 9 aa, Artificial Sequence
  Synthetic Polypeptide
QAWDSTTVV

SEQ ID NO: 83 - protein, 121 aa, Artificial Sequence
  Synthetic Polypeptide
QLQLQQSGGGLVKPGGSLRLSCAASGFTFSSYSMNWVRQAPGKGLEWVSSISSSSSYIYYADSVKGRFTISRDNAKNSLYLQMNSLRAEDTAVYYCVRDRHSLGDFDYWGQGTLVTVSSGS

SEQ ID NO: 84 - protein, 121 aa, Artificial Sequence
  Synthetic Polypeptide
SSELTQPSVSVSPGQTATITCSGDKLGDKYASWYQQKPGQSPVLVIYQDTKRPSGIPARFSGSNSGNTATLTISGTQAMDEAAYYCQAWDSTTVVFGGGTKLTVLGQPKAAPSVTLFPPSS

SEQ ID NO: 85 - protein, 201 aa, Artificial Sequence
  Synthetic Polypeptide
QLQLQQSGGGLVKPGGSLRLSCAASGFTFSSYSMNWVRQAPGKGLEWVSSISSSSSYIYYADSVKGRFTISRDNAKNSLYLQMNSLRAEDTAVYYCVRDRHSLGDFDYWGQGTLVTVSSGSASAPTLGGGGSGGGGSAAASSELTQPPSVSVSPGQTATITCSGDKLGDKYASWYQQKPGQSPVLVIYQDTKRPSGIPARF

SEQ ID NO: 86 - protein, 20 aa, Artificial Sequence
  Synthetic Polypeptide
ANHGLMDDSSGYYLSNAFDI

SEQ ID NO: 87 - protein, 11 aa, Artificial Sequence
  Synthetic Polypeptide
ATWDDSLTGVV

SEQ ID NO: 88 - protein, 129 aa, Artificial Sequence
  Synthetic Polypeptide
QVQLVQSGAEVKKPGSSVKVSCKASGGTFSSYAISWVRQAPGQGLEWMGGIIPIFGTANYAQKFQGRVTITADESTSTAYMELSSLRSEDTAVYYCANHGLMDDSSGYYLSNAFDIWGQGTMVTVSSGS

SEQ ID NO: 89 - protein, 126 aa, Artificial Sequence
  Synthetic Polypeptide
QPVLTQPPSASGTPGQRVTISCSGSSSNIGSNTVEWYQQLPGTAPKLLIHSNNQRPSGVPDRFSGSRSGTSASLAISGLQSEDEADYFCATWDDSLTGVVFGGGTTLTVLGQPKAAPSVTLFPPSS

SEQ ID NO: 90 - protein, 274 aa, Artificial Sequence
  Synthetic Polypeptide
QVQLVQSGAEVKKPGSSVKVSCKASGGTFSSYAISWVRQAPGQGLEWMGGIIPIFGTANYAQKFQGRVTITADESTSTAYMELSSLRSEDTAVYYCANHGLMDDSSGYYLSNAFDIWGQGTMVTVSSGSASAPTLGGGGSGGGGSAAAQPVLTQPPSASGTPGQRVTISCSGSSSNIGSNTVEWYQQLPGTAPKLLIHSNNQRPSGVPDRFSGSRSGTSASLAISGLQSEDEADYFCATWDDSLTGVVFGGGTTLTVLGQPKAAPSVTLFPPSS

SEQ ID NO: 91 - protein, 14 aa, Artificial Sequence
  Synthetic Polypeptide
AKVGTAAAGDAFDI

SEQ ID NO: 92 - protein, 11 aa, Artificial Sequence
  Synthetic Polypeptide
AAWDDSLSGWV

SEQ ID NO: 93 - protein, 123 aa, Artificial Sequence
  Synthetic Polypeptide
QVQLVQSGGGLIQPGGSLRLSCAASGFTVSSYSMNWVRQAPGKGLEWVSYISSSGSTIYYADSVKGRFTISRDNAKNSLYLQMNSLRAEDTALYYCAKVGTAAAGDAFDIWGQGTMVTVSSGS

SEQ ID NO: 94 - protein, 126 aa, Artificial Sequence
  Synthetic Polypeptide
QPVLTQPPSASGTPGQRVTISCFGSSSNIGSNYVYWYQQLPGTAPKLLIYRNNQRPSGVPDRFSGSKSGTSASLAISGLRSEDEADYYCAAWDDSLSGWVFGGGTKLTVLGQPKAAPSVTLFPPSS

SEQ ID NO: 95 - protein, 268 aa, Artificial Sequence
  Synthetic Polypeptide
QVQLVQSGGGLIQPGGSLRLSCAASGFTVSSYSMNWVRQAPGKGLEWVSYISSSGSTIYYADSVKGRFTISRDNAKNSLYLQMNSLRAEDTALYYCAKVGTAAAGDAFDIWGQGTMVTVSSGSASAPTLGGGGSGGGGSAAAQPVLTQPPSASGTPGQRVTISCFGSSSNIGSNYVYWYQQLPGTAPKLLIYRNNQRPSGVPDRFSGSKSGTSASLAISGLRSEDEADYYCAAWDDSLSGWVFGGGTKLTVLGQPKAAPSVTLFPPSS

SEQ ID NO: 96 - protein, 20 aa, Artificial Sequence
  Synthetic Polypeptide
ARVGFYDYVWGSYPYDAFDI

SEQ ID NO: 97 - protein, 9 aa, Artificial Sequence
  Synthetic Polypeptide
QQYGTSPLT

SEQ ID NO: 98 - protein, 129 aa, Artificial Sequence
  Synthetic Polypeptide
QIQLVQSGAEVKKPGASVKVSCKASGYTFTSYGISWVRQAPGQGLEWMGWISAYNGNTNYAQKLQGRVTMTTDTSTSTAYMELSSLRSEDTAVYYCARVGFYDYVWGSYPYDAFDIWGQGTMVTVSSGS

SEQ ID NO: 99 - protein, 117 aa, Artificial Sequence
  Synthetic Polypeptide
EIVMTQSPGTLSLSPGERATLSCRASQSVSSNYLAWYQQKPGQAPRLLIYDASNRATGIPARFSGSGSGTDFTLTISSLEPEDFALYYCQQYGTSPLTFGGGTKLEIKRTVAAPSVF

SEQ ID NO: 100 - protein, 265 aa, Artificial Sequence
  Synthetic Polypeptide
QIQLVQSGAEVKKPGASVKVSCKASGYTFTSYGISWVRQAPGQGLEWMGWISAYNGNTNYAQKLQGRVTMTTDTSTSTAYMELSSLRSEDTAVYYCARVGFYDYVWGSYPYDAFDIWGQGTMVTVSSGSASAPTLGGGGSGGGGSAAAEIVMTQSPGTLSLSPGERATLSCRASQSVSSNYLAWYQQKPGQAPRLLIYDASNRATGIPARFSGSGSGTDFTLTISSLEPEDFALYYCQQYGTSPLTFGGGTKLEIKRTVAAPSVF

SEQ ID NO: 101 - protein, 16 aa, Artificial Sequence
  Synthetic Polypeptide
AKDTSNGGYSSSSFDY

SEQ ID NO: 102 - protein, 10 aa, Artificial Sequence
  Synthetic Polypeptide
SSYTSSSTLV

SEQ ID NO: 103 - protein, 125 aa, Artificial Sequence
  Synthetic Polypeptide
EVQLVQSGGGLVQPGRSLRLSCAASGFTFDDYAMHWVRQAPGKGLEWVSGISWNSGSIGYADSVKGRFTISRDNAKNSLYLQMNSLRAEDTALYYCAKDTSNGGYSSSSFDYWGQGTLVTVSSGS

SEQ ID NO: 104 - protein, 126 aa, Artificial Sequence
  Synthetic Polypeptide
QSALTQPASVSGSPGQSITISCTGTSSDVGGYNYVSWYQQHPGTAPKLMIYDVSYRPSGVSNRFSGSKSGNTASLTISGLQAEDEADYYCSSYTSSSTLVFGTGTKVTVLGQPKANPTVTLFPPSS

SEQ ID NO: 105 - protein, 270 aa, Artificial Sequence
  Synthetic Polypeptide
EVQLVQSGGGLVQPGRSLRLSCAASGFTFDDYAMHWVRQAPGKGLEWVSGISWNSGSIGYADSVKGRFTISRDNAKNSLYLQMNSLRAEDTALYYCAKDTSNGGYSSSSFDYWGQGTLVTVSSGSASAPTLGGGGSGGGGSAAAQSALTQPASVSGSPGQSITISCTGTSSDVGGYNYVSWYQQHPGTAPKLMIYDVSYRPSGVSNRFSGSKSGNTASLTISGLQAEDEADYYCSSYTSSSTLVFGTGTKVTVLGQPKANPTVTLFPPSS

SEQ ID NO: 106 - protein, 17 aa, Artificial Sequence
  Synthetic Polypeptide
ARLVYGGYDEPGYYFDY

SEQ ID NO: 107 - protein, 11 aa, Artificial Sequence
  Synthetic Polypeptide
AAWDDSLNGWV

SEQ ID NO: 108 - protein, 126 aa, Artificial Sequence
  Synthetic Polypeptide
EVQLLESRAEVKKPGESLKISCKGSGYSFTSYWIGWVRQMPGKGPEWMGIIYPGDSDTRYSPSFQGQVTISADKSISTAYLQWSSLKASDTAMYYCARLVYGGYDEPGYYFDYWGQGTLVTVSSGS

SEQ ID NO: 109 - protein, 131 aa, Artificial Sequence
  Synthetic Polypeptide
QSVLTQPPSASGTPGQRVTISCSGSSSNIRSNTVNWYQQLPGTAPKLLIYSNNQRPSGVPDRFSGSKSGTSASLAISGLQSEDEADYYCAAWDDSLNGWVFGGGTKLTVLGQPKAAPSVTLFPPSSKASGA

SEQ ID NO: 110 - protein, 276 aa, Artificial Sequence
  Synthetic Polypeptide
EVQLLESRAEVKKPGESLKISCKGSGYSFTSYWIGWVRQMPGKGPEWMGIIYPGDSDTRYSPSFQGQVTISADKSISTAYLQWSSLKASDTAMYYCARLVYGGYDEPGYYFDYWGQGTLVTVSSGSASAPTLGGGGSGGGGSAAAQSVLTQPPSASGTPGQRVTISCSGSSSNIRSNTVNWYQQLPGTAPKLLIYSNNQRPSGVPDRFSGSKSGTSASLAISGLQSEDEADYYCAAWDDSLNGWVFGGGTKLTVLGQPKAAPSVTLFPPSSKASGA

SEQ ID NO: 111 - protein, 16 aa, Artificial Sequence
  Synthetic Polypeptide
AKVDGLEYSSGHNFDY

SEQ ID NO: 112 - protein, 10 aa, Artificial Sequence
  Synthetic Polypeptide
SSYAGSYTWV

SEQ ID NO: 113 - protein, 125 aa, Artificial Sequence
  Synthetic Polypeptide
EVQLVQSGGGLVQPGRSLRLSCAASGFTFDDYAMHWVRQAPGKGLEWVSGISWNSGSIGYADSVKGRFTISRDNSKNTLYLQMNSLRAEDTAVYYCAKVDGLEYSSGHNFDYWGQGTLVTVSSGS

SEQ ID NO: 114 - protein, 126 aa, Artificial Sequence
  Synthetic Polypeptide
QSALTQPPSVSGSPGQSVTISCTGSSSDVGYYDHVSWYQHHPGRAPKVIIYDVTKRPSGVPDRFSGSKSGNTASLTISGLQAEDEADYYCSSYAGSYTWVFGGGTELTVLGQPKAAPSVTLFPPSS

SEQ ID NO: 115 - protein, 270 aa, Artificial Sequence
  Synthetic Polypeptide
EVQLVQSGGGLVQPGRSLRLSCAASGFTFDDYAMHWVRQAPGKGLEWVSGISWNSGSIGYADSVKGRFTISRDNSKNTLYLQMNSLRAEDTAVYYCAKVDGLEYSSGHNFDYWGQGTLVTVSSGSASAPTLGGGGSGGGGSAAAQSALTQPPSVSGSPGQSVTISCTGSSSDVGYYDHVSWYQHHPGRAPKVIIYDVTKRPSGVPDRFSGSKSGNTASLTISGLQAEDEADYYCSSYAGSYTWVFGGGTELTVLGQPKAAPSVTLFPPSS

SEQ ID NO: 116 - protein, 323 aa, Artificial Sequence
  Synthetic Polypeptide
ASTTPPSVYPLAPGSAAQTNSMVTLGCLVKGYFPEPVTVTWNSGSLSSGVHTFPAVLQSDLYTLSSSVTVPSSTWPSETVTCNVAHPASSTKVDKKIVPRDCGCKPCICTVPEVSSVFIFPPKPKDVLTITLTPKVTCVVVDISKDDPEVQFSWFVDDVEVHTAQTQPREEQFNSTFRSVSELPIMHQDWLNGKEFKCRVNSAAFPAPIEKTISKTKGRPKAPQVYTIPPPKEQMAKDKVSLTCMITDFFPEDITVEWQWNGQPAENYKNTQPIMDTDGSYFVYSKLNVQKSNWEAGNTFTCSVLHEGLHNHHTEKSLSHSPG

SEQ ID NO: 117 - protein, 106 aa, Artificial Sequence
  Synthetic Polypeptide
GQPKSSPSVTLFPPSSEELETNKATLVCTITDFYPGVVTVDWKVDGTPVTQGMETTQPSKQSNNKYMASSYLTLTARAWERHSSYSCQVTHEGHTVEKSLSRADCS

SEQ ID NO: 118 - protein, 6 aa, Artificial Sequence
  Synthetic Polypeptide
KALDEN